European Patent Application EP 4 756 035 A1, published June 10, 2026. Title: METHOD FOR PURIFYING NUCLEIC ACID AND KIT FOR PURIFYING NUCLEIC ACID. Applicant: 栄研化学株式会社. The sequence listing filed with the application follows.

SEQUENCE LISTING (12 sequences)

SEQ ID NO: 1 - DNA, 20 bp, synthetic construct
  source 1..20: mol_type = other DNA
aaattttggggaccaggaac

SEQ ID NO: 2 - DNA, 20 bp, synthetic construct
  source 1..20: mol_type = other DNA
tggcagctgtgtaggtcaac

SEQ ID NO: 3 - DNA, 20 bp, synthetic construct
  source 1..20: mol_type = other DNA
atgtcgcgcattggcatgga

SEQ ID NO: 4 - DNA, 20 bp, synthetic construct
  source 1..20: mol_type = other DNA
ggactctggacatgcaagat

SEQ ID NO: 5 - DNA, 21 bp, synthetic construct
  source 1..21: mol_type = other DNA
atacccttcttaacacctggc

SEQ ID NO: 6 - DNA, 30 bp, synthetic construct
  source 1..30: mol_type = other DNA
cccttcagagcgttttctctaaattgatac

SEQ ID NO: 7 - DNA, 21 bp, synthetic construct
  source 1..21: mol_type = other DNA
acgcaatctagcagatgaagc

SEQ ID NO: 8 - DNA, 21 bp, synthetic construct
  source 1..21: mol_type = other DNA
tgtttggttggttattcgtgc

SEQ ID NO: 9 - DNA, 25 bp, synthetic construct
  source 1..25: mol_type = other DNA
tttgccgaaaacgcttgatacaggg

SEQ ID NO: 10 - DNA, 29 bp, synthetic construct
  source 1..29: mol_type = other DNA
ccmaggtcgaaacgtaygttctctctatc

SEQ ID NO: 11 - DNA, 32 bp, synthetic construct
  source 1..32: mol_type = other DNA
tgacagratyggtcttgtctttagccaytcca

SEQ ID NO: 12 - DNA, 23 bp, synthetic construct
  source 1..23: mol_type = other DNA
cagccagcaatrttrcatttacc